European Patent Specification EP 3 255 140 B1, published October 16, 2024. Title: Lactic acid bacterium, innate immunity activator derived therefrom, agent for preventing or treating infection, and food and drink. Applicant: Genome Pharmaceuticals Institute Co., Ltd. Antenna Co., Ltd. The University of Tokyo. The sequence listing filed with the application follows.

SEQUENCE LISTING (1 sequence)

SEQ ID NO: 1 - DNA, 1480 bp, Lactobacillus paraplantarum
  misc_feature (4)..(6): n is a, c, g, or t
  misc_feature (1473)..(1473): n is a, c, g, or t
ctannntgcaagtcgaacgaactctggttaatgattgaaggtgcttgcacctgattgatttaacatttgagtgagtggcgaactggtgagtaacacgtgggaaacctgcccagaagtgggggataacacctggaaacagatgctaataccgcataacaactcggaccgcatggtctgagtttaaaagatggcttcggctatcacttttggatggtcccgcggcgtattagctagatggtgaggtaacggctcaccatggcaatgatacgtagccgacctgagagggtaatcggccacattgggactgagacacggcccaaactcctacgggaggcagcagtagggaatcttccacaatggacgaaagtctgatggagcaacgccgcgtgagtgaagaagggtttcggctcgtaaaactctgttgttaaagaagaacatatctgagagtaactgttcaggtattgacggtatttaaccagaaagccacggctaactacgtgccagcagccgcggtaatacgtaggtggcaagcgttatccggatttattgggcgtaaagcgagcgcaggcggttttttaagtctgatgtgaaagccttcggctcaaccgaagaagtgcatcggaaactgggaaacttgagtgcagaaaaggacagtggaactccatgtgtagcggtgaaatgcgtagatatatggaagaacaccagtggcgaaggcggctgtctggtctgtaactgacgctgaggctcgaaagtatgggtagcaaacaggattagataccctggtagtccataccgtaaacgatgaatgctaagtgttggagggtttccgcccttcagtgctgcagctaacgcattaagcattccgcctggggagtacggccgcaaggctgaaactcaaaggaattgacgggggcccgcacaagcggtggagcatgtggtttaattcgaagctacgcgaagaaccttaccaggtcttgacatactatgcaaatctaagagattagacgttcccttcggggacatggatacaggtggtgcatggttgtcgtcagctcgtgtcgtgagatgttgggttaagtcccgcaacgagcgcaacccttattattagttgccagcattaagttgggcactctagtgagactgccggtgacaaaccggaggaaggtggggatgacgtcaaatcatcatgccccttatgacctgggctacacacgtgctacaatggatggtacaacgagttgcgaactcgcgagagtaagctaatctcttaaagccattctcagttcggattgtaggctgcaactcgcctacatgaagtcggaatcgctagtaatcgcggatcagcatgccgcggtgaatacgttcccgggccttgtacacaccgcccgtcacaccatgagagtttgtaacacccaaagtcggtggggtaaccttcggggaccagccgcctaaggtgggacagatgattagggngaagtcg